European Patent Application EP 4 257 597 A1, published October 11, 2023. Title: LACTAM-MODIFIED POLYPEPTIDE COMPOUNDS. Applicant: DONGBAO PURPLE STAR (HANGZHOU) BIOPHARMACEUTICAL CO., LTD. The sequence listing filed with the application follows.

SEQUENCE LISTING (4 sequences)

SEQ ID NO: 1 - protein, 39 aa, Artificial Sequence
  Compound
  MISC_FEATURE (2)..(2): X is Aib in the description
  MISC_FEATURE (13)..(13): X is Aib in the description
  MISC_FEATURE (17)..(17): K is K1 in the description, K1 indicates that the amino group on the side chain of the lysine is connected to -X-X1-X2
  MISC_FEATURE (19)..(19): X is Z0 in the description, Z0 is selected from glutamine (Q) and asparagine (N)
  MISC_FEATURE (20)..(20): K is K0 in the description, K0 indicates that the carboxyl group on the side chain of the glutamic acid (E0) and the amino group on the side chain of the lysine (K0) jointly form a lactam structure
  MISC_FEATURE (21)..(21): X is Z1 in the descriptionZ1 is selected from alanine (A) and glutamic acid (E)
  MISC_FEATURE (23)..(23): X is Z2 in the description, Z2 is selected from valine (V) and isoleucine (I)
  MISC_FEATURE (24)..(24): E is E0 in the description, E0 indicates that the carboxyl group on the side chain of the glutamic acid (E0) and the amino group on the side chain of the lysine (K0) jointly form a lactam structure
  MISC_FEATURE (27)..(27): X is Z3 in the description, Z3 is selected from isoleucine (I) and leucine (L)
  MISC_FEATURE (39)..(39): S is S0 in the description
YXEGTFTSDYSIXLDKKAXKXFXEWLXAGGPSSGAPPPS

SEQ ID NO: 2 - protein, 39 aa, Artificial Sequence
  Compound
  MISC_FEATURE (2)..(2): X is Aib in the description
  MISC_FEATURE (13)..(13): X is Aib in the description
  MISC_FEATURE (17)..(17): E is E0 in the description, E0 indicates that the carboxyl group on the side chain of the glutamic acid (E0) and the amino group on the side chain of the lysine (K0) jointly form a lactam structure
  MISC_FEATURE (20)..(20): K is K0 in the description, K0 indicates that the carboxyl group on the side chain of the glutamic acid (E0) and the amino group on the side chain of the lysine (K0) jointly form a lactam structure
  MISC_FEATURE (24)..(24): K is K1 in the description, K1 indicates that the amino group on the side chain of the lysine is connected to -X-X1-X2
  MISC_FEATURE (39)..(39): S is S0 in the description
YXEGTFTSDYSIXLDKEAQKAFVKWLIAGGPSSGAPPPS

SEQ ID NO: 3 - protein, 39 aa, Artificial Sequence
  Compound
  MISC_FEATURE (2)..(2): X is Aib in the description
  MISC_FEATURE (13)..(13): E is E0 in the description, E0 indicates that the carboxyl group on the side chain of the glutamic acid (E0) and the amino group on the side chain of the lysine (K0) jointly form a lactam structure
  MISC_FEATURE (17)..(17): K is K0 in the description, K0 indicates that the carboxyl group on the side chain of the glutamic acid (E0) and the amino group on the side chain of the lysine (K0) jointly form a lactam structure
  MISC_FEATURE (20)..(20): K is K1 in the description, K1 indicates that the amino group on the side chain of the lysine is connected to -X-X1-X2
  MISC_FEATURE (39)..(39): S is S0 in the description
YXEGTFTSDYSIELDKKAQKAFVQWLIAGGPSSGAPPPS

SEQ ID NO: 4 - protein, 39 aa, Artificial Sequence
  Compound
  MISC_FEATURE (2)..(2): X is Aib in the description
  MISC_FEATURE (13)..(13): E is E0 in the description, E0 indicates that the carboxyl group on the side chain of the glutamic acid (E0) and the amino group on the side chain of the lysine (K0) jointly form a lactam structure
  MISC_FEATURE (16)..(16): K is K0 in the description, K0 indicates that the carboxyl group on the side chain of the glutamic acid (E0) and the amino group on the side chain of the lysine (K0) jointly form a lactam structure
  MISC_FEATURE (20)..(20): K is K1 in the description, K1 indicates that the amino group on the side chain of the lysine is connected to -X-X1-X2
  MISC_FEATURE (39)..(39): S is S0 in the description
YXEGTFTSDYSIELDKIAQKAFVQWLIAGGPSSGAPPPS